European Patent Specification EP 3 336 194 B1, published January 10, 2024. Title: 3-epimerase. Applicant: Tate & Lyle Technology Limited. The sequence listing filed with the application follows.

SEQUENCE LISTING (15 sequences)

SEQ ID NO: 1 - DNA, 903 bp, Clostridium scindens
  CDS (4)..(888)
catatgaatcgtattggcatttttatgaatttttgggtgaagaactgggacgctgaccacgttaagtacatcaagaaggtgtcgggcctgggctttgatattctggaatttcaggcacaagctctgctggaaatggataaatctcgtatggacgaagtgcgccaggcggccaaggataacggcattgaactgacctattctctgggtctgaatccgaaatacgatgtggcaagtccggacgctaaggttcgtgaaggcggtatcgaatatctgaaacgtattgtggaacgcatcggctacatggaaggcaagctgctgtcaggcgttaactatgcgggctggggttcgccggattacattgtcgatgacaaaagcgaaattgtggaacatagcatcgaaagcgtgcgtcaggtcatcaaaaccgccgaagattatgacgtgacgtactgcgttgaagtggttaaccgctttgaaggcattgttatgaataccgcgaaagaagccattgaatatgtcaaacaaatcgatagcgacaagattggtatcctgctggatacgtaccacatgaacatcgaagaaggcagtattggtgatgcgatccgttccgttggcggttatctgaaaaatttccacacgggcgaaaacaatcgcgtcgtgccgggcaagggtcatctggattgggacgaaatttttggcgcactgcacgatattgactaccagggtcgcatcgtctccgaaccgttcgtgcaaatgggcggtgaagtggctcgtgatatcaaagtttggcgcgatctggtcgaagacccgagcgaagaagttctggatgaagaagcgcgttttctgctgaatttcgaaaaagacatgattcgcaagcactatggtatcgcctaaagatctggatcc

SEQ ID NO: 2 - protein, 295 aa, Clostridium scindens
MNRIGIFMNFWVKNWDADHVKYIKKVSGLGFDILEFQAQALLEMDKSRMDEVRQAAKDNGIELTYSLGLNPKYDVASPDAKVREGGIEYLKRIVERIGYMEGKLLSGVNYAGWGSPDYIVDDKSEIVEHSIESVRQVIKTAEDYDVTYCVEVVNRFEGIVMNTAKEAIEYVKQIDSDKIGILLDTYHMNIEEGSIGDAIRSVGGYLKNFHTGENNRVVPGKGHLDWDEIFGALHDIDYQGRIVSEPFVQMGGEVARDIKVWRDLVEDPSEEVLDEEARFLLNFEKDMIRKHYGIA

SEQ ID NO: 3 - DNA, 885 bp, Clostridium hylemonae
  CDS (4)..(870)
catatgaaacacggtatctattacgcctattgggaacaagaatgggcagcagactacaaacgctatgtggaaaaagtggcaaaactgggcttcgatattctggaaatcggcgccggtccgctgccggaatatgcagaacaggacgttaaagaactgaaaaagtgcgctcaagataacggcattaccctgacggcgggctacggtccgacctttaaccataatatcggcagctctgatgctggtgtgcgtgaagaagcgctggaatggtataaacgcctgttcgaagttctggccgaactggacattcacctgatcggcggtgcactgtatagttactggccggtcgattttgctaacgcggacaaaacggaagattggaagtggtccgtggagggtatgcagcgtctggccccggcggcggcaaaatacgatattaacctgggtatggaagttctgaatcgctttgaatcacatatcctgaataccgccgaagaaggcgtcaaattcgtggaagaagttggtatggacaacgtgaaggttatgctggatacgttccacatgaatattgaagaacaatcgattggcggtgccatccgtcgcgcaggcaaactgctgggtcattttcacaccggcgaatgtaatcgtatggtgccgggcaagggtcgtattccgtggcgcgaaatcggtgacgctctgcgtgatatcggctacgacggtacggcagtcatggaaccgttcgtgcgtatgggtggtcaggttggtgcagatattaaagtctggcgtgacatctctcgcggtgccgatgaagcacagctggatgacgatgctcgtcgcgcgctggaatttcaacgctatatgctggaatggaagtaaagatctggatcc

SEQ ID NO: 4 - protein, 289 aa, Clostridium hylemonae
MKHGIYYAYWEQEWAADYKRYVEKVAKLGFDILEIGAGPLPEYAEQDVKELKKCAQDNGITLTAGYGPTFNHNIGSSDAGVREEALEWYKRLFEVLAELDIHLIGGALYSYWPVDFANADKTEDWKWSVEGMQRLAPAAAKYDINLGMEVLNRFESHILNTAEEGVKFVEEVGMDNVKVMLDTFHMNIEEQSIGGAIRRAGKLLGHFHTGECNRMVPGKGRIPWREIGDALRDIGYDGTAVMEPFVRMGGQVGADIKVWRDISRGADEAQLDDDARRALEFQRYMLEWK

SEQ ID NO: 5 - DNA, 885 bp, Desmospora sp.8437
  CDS (4)..(870)
catatgaaatacggtgtctactttgcttactgggaagattcgtgggatgttgactttgaaaaatacgttcgcaaggtgaaaaaactgggctttgatattctggaagttgcagcactgggtctggtcaacctgccggaagaaaaactggaacgtctgaagcagctggcggaacaacatgacattatcctgaccgccggcattggtctgccgaaagaatatgatgtcagctctacggacaaaaaagtgcgtcgcaatggcatctcctttatgaaaaaggttatggatgcaatgcatcaggctggtattcaccgtattggcggcaccgtgtatagctactggccggttgattacagttgctccttcgacaaaccggcggttcgcaagcactcaattgaatcggtccgtgaactggcggaatatgcccgccagtacaacattaccctgctgatcgaaacgctgaaccgctttgaacaattcctgctgaatgatgccgaagaagcggttgcctatgtcaaagaagtggatgaaccgaacgtcaaggtgatgctggacaccttccacatgaacatcgaagaagatcacatcgcagacgctatccgttacacgggcgatcatctgggtcagctgcacatcggcgaagccaaccgcaaagtgccgggcaagggtagtatgccgtggaccgaaattggccaagcactgaaagatatccgttatgacggttacgtggttatggaaccgttcattaaaaccggcggtcaggttggccgtgatatcaaactgtggcgcgacctgagcggtaatgcaacggaagaacaactggatcgcgaactggctgaatctctggaatttgtgaaagcagctttcggtgaataaagatctggatcc

SEQ ID NO: 6 - protein, 289 aa, Desmospora sp.8437
MKYGVYFAYWEDSWDVDFEKYVRKVKKLGFDILEVAALGLVNLPEEKLERLKQLAEQHDIILTAGIGLPKEYDVSSTDKKVRRNGISFMKKVMDAMHQAGIHRIGGTVYSYWPVDYSCSFDKPAVRKHSIESVRELAEYARQYNITLLIETLNRFEQFLLNDAEEAVAYVKEVDEPNVKVMLDTFHMNIEEDHIADAIRYTGDHLGQLHIGEANRKVPGKGSMPWTEIGQALKDIRYDGYVVMEPFIKTGGQVGRDIKLWRDLSGNATEEQLDRELAESLEFVKAAFGE

SEQ ID NO: 7 - DNA, 897 bp, Clostridium cellulolyticum
  CDS (4)..(882)
catatgaagcacggcatctattacgcctattgggaacaagaatgggaagcagactacaagtattacatcgaaaaggttgcgaagctgggttttgatattctggaaatcgcggcctcaccgctgccgttttattcggacattcagatcaatgaactgaaagcgtgcgcgcatggcaacggtattaccctgacggtgggccacggtccgagcgcggaacaaaatctgagcagcccggacccggacatccgtaaaaacgcaaaggctttctataccgatctgctgaaacgcctgtacaagctggacgttcatctgattggcggtgccctgtattcttactggccgatcgattacaccaagacgatcgataagaagggcgactgggaacgtagtgttgaatccgtccgcgaagtggccaaggttgcggaagcctgcggtgtcgatttttgtctggaagtgctgaaccgtttcgaaaattacctgattaacaccgcacaggaaggcgtcgattttgtgaaacaagttgaccataacaatgtcaaggtgatgctggatacgttccacatgaatatcgaagaagacagtattggcggtgcgatccgtaccgccggctcctatctgggtcatctgcacacgggcgaatgcaatcgcaaagttccgggccgtggtcgcattccgtgggtcgaaatcggtgaagcactggctgatattggctacaacggttcagtggttatggaaccgtttgttcgtatgggcggcaccgtcggcagcaatattaaagtgtggcgcgatatctctaacggtgcagatgaaaagatgctggaccgtgaagctcaggcagctctggacttctcacgctacgtgctggaatgtcataaacactcgtaaagatctggatcc

SEQ ID NO: 8 - protein, 293 aa, Clostridium cellulolyticum
MKHGIYYAYWEQEWEADYKYYIEKVAKLGFDILEIAASPLPFYSDIQINELKACAHGNGITLTVGHGPSAEQNLSSPDPDIRKNAKAFYTDLLKRLYKLDVHLIGGALYSYWPIDYTKTIDKKGDWERSVESVREVAKVAEACGVDFCLEVLNRFENYLINTAQEGVDFVKQVDHNNVKVMLDTFHMNIEEDSIGGAIRTAGSYLGHLHTGECNRKVPGRGRIPWVEIGEALADIGYNGSVVMEPFVRMGGTVGSNIKVWRDISNGADEKMLDREAQAALDFSRYVLECHKHS

SEQ ID NO: 9 - DNA, 885 bp, Clostridium scindens
aacagaataggaatatttatgaatttctgggttaagaactgggatgcagatcatgtcaagtatattaaaaaggtatccggccttggatttgatattctggaattccaggcccaggcgcttctggagatggataagagcaggatggatgaggtcaggcaggcggcaaaggacaatggaatcgaactgacctacagccttgggctgaatcctaagtacgatgtcgcaagcccggatgcaaaagtcagggaaggcggaatcgaatatctgaagcggatcgtggagcggattggatacatggaaggaaaactgctttccggagtcaactatgccggctggggaagcccggactatatcgtggatgacaaaagcgagatcgtggagcacagcatcgaaagcgtccgccaggtcattaagacggcagaagattatgacgtgacttactgcgtggaggtcgtgaaccggtttgagggcatcgtgatgaatacggcaaaggaagccatcgagtacgtgaagcagattgacagtgataagatcggaatcctgctggatacctatcatatgaacatcgaggaaggctctataggagacgccatccgatctgtaggcggatatctgaagaacttccacactggagagaacaaccgggtcgttccggggaaggggcacctcgactgggatgaaatatttggagcgctccatgatatcgattatcagggaaggatcgtgtcagagccgttcgtccagatgggcggggaagtcgcaagagacatcaaggtatggagagatctggtggaagatccttcagaagaagtgctggatgaggaggcgcgcttccttctgaattttgaaaaggatatgatccggaagcactatggcatagcgtaa

SEQ ID NO: 10 - DNA, 867 bp, Clostridium hylemonae
aaacatggtatctattatgcatactgggaacaagaatgggcggccgactacaagcgctatgttgaaaaggtggcaaagcttgggtttgacattctggagatcggcgctgggccgctgccggaatacgcagagcaggatgtgaaggaactgaagaaatgtgcgcaggacaatgggatcacgctgacggccggatatggtccgacgttcaaccacaatatcggttcttcagacgccggggtaagggaagaggcgctggaatggtataagaggttatttgaagtgctggcagagcttgatatccacctgatcggaggggcgctctattcttactggcctgtcgattttgcaaacgccgataaaacggaagactggaagtggagtgtagagggcatgcagaggctggcgccggccgcggccaaatatgacatcaacctgggcatggaagttctgaaccggtttgagagccatatcctgaatacagccgaggaaggtgtgaagtttgtagaggaagtcggcatggacaacgtaaaggtcatgctggatacattccatatgaatatagaagagcaaagcataggcggcgcgatccgccgggcaggaaaactgctcgggcatttccacaccggagaatgcaaccgcatggtgcccgggaagggacgtattccatggcgtgagataggggatgctctccgtgatatcggatatgacggaactgctgtaatggagccgttcgttcgcatgggaggacaggtcggcgctgatatcaaggtgtggagagacataagccgtggagcagacgaggcacagcttgacgatgacgcgcgccgtgcgctggagttccagagatatatgctggagtggaagtaa

SEQ ID NO: 11 - DNA, 867 bp, Desmospora sp
aaatacggtgtctatttcgcttactgggaagactcgtgggatgtggatttcgagaagtacgtgcggaaagtgaaaaagttgggcttcgacatcctcgaagtggcggcattgggtctcgtcaaccttccggaggagaaactggagcggctgaaacaactcgccgaacagcacgatatcatcctgacggccgggatcggcctgccaaaggaatacgatgtctcgtcaactgacaaaaaggtgcgccggaacggcatctccttcatgaagaaagtgatggacgcgatgcatcaggccggcatccaccggatcggcggcacggtctactcgtattggccggttgactacagttgctccttcgacaagccggccgtaaggaagcacagcatcgaaagcgtcagagagctggcggagtacgcacggcagtacaacatcacactcctcatcgaaacgctcaaccggtttgagcagtttctcctgaacgacgcggaggaagcagtcgcctatgtgaaggaagtggacgagccgaatgtgaaagtcatgctcgacacattccacatgaacatcgaggaagaccacattgccgatgccatccgctacaccggtgaccacctcggccaactgcacatcggcgaagcgaatcggaaagtcccgggcaagggttcgatgccttggacagaaatcggacaggcgctgaaagacattcgctacgatggctacgttgtcatggaacccttcatcaaaaccggcggacaggtcggccgggacatcaagctctggcgcgatctgtcgggaaatgcgacggaggaacagttggaccgggagctggcagagtcgctggaatttgtgaaagcggcgttcggggagtaa

SEQ ID NO: 12 - DNA, 879 bp, Clostridium cellulolyticum
aaacatggtatatactacgcatattgggaacaagaatgggaagctgattacaaatactatattgagaaggttgcaaagcttggttttgatattctagagattgcagcttcaccgctacctttttacagtgacattcagattaatgagctcaaggcatgtgcccatggcaatggaattacacttacggtaggccatgggcctagtgcagaacaaaacctgtcttctcccgaccccgatattcgcaaaaatgctaaagctttttataccgatttactcaaacgactttacaagctggatgtacatttgataggtggggctttatattcttattggccgatagattacacaaagacaattgataaaaaaggcgattgggaacgcagcgttgaaagtgttcgagaagttgctaaggtggccgaagcctgtggagtggatttctgcctagaggttcttaatagatttgagaattatttaattaacacagcacaagagggtgtagattttgtaaaacaggttgaccataacaatgtaaaggtaatgcttgataccttccatatgaatattgaggaagatagtatcggaggtgcaatcaggactgcgggctcttacttgggacatttacacactggcgaatgtaatcgtaaagttcccggcagaggaagaattccatgggtagaaattggtgaggctcttgctgacataggttataacggtagtgttgttatggaaccttttgttagaatgggcggaactgtcggatctaatattaaggtttggcgtgacattagtaacggtgcagatgagaaaatgctggatagagaagcacaggccgcacttgatttctccagatatgtattagaatgtcataaacactcctga

SEQ ID NO: 13 - protein, 289 aa, Artificial Sequence
  Artificial variant of the ketose-3-epimerase of Desmospora sp. 8437.
MRYGIYYAYWEDSWDADFEKYVKKVKKLGFDIIEVAALGFVNLPEEKLETLRQLAEQHDIILTAGYGLPKEYNVSSPDKKVRRNGISFMKKVLDAMHQLGIHRIGGTVFSYWPVDYSCSFDKPAVRKHAIESVREVAEYARQYNITLAIEVLNRFEQFVLNDAEEAIAYVKEVGEPNVKVMLDTFHMNIEEDHFADAIRYAGDLLGQLHIGEANRKVPGKGSLPWTEIGQALKDIRYDGYVIMEPFVKTGGTVGRDVKLWRDMSGNATEEQLDRELAESLEFVRAAFGE

SEQ ID NO: 14 - protein, 289 aa, Agrobacterium tumefaciens
MKHGIYYSYWEHEWSAKFGPYIEKVAKLGFDIIEVAAHHINEYSDAELATIRKSAKDNGIILTAGIGPSKTKNLSSEDAAVRAAGKAFFERTLSNVAKLDIHTIGGALHSYWPIDYSQPVDKAGDYARGVEGINGIADFANDLGINLCIEVLNRFENHVLNTAAEGVAFVKDVGKNNVKVMLDTFHMNIEEDSFGDAIRTAGPLLGHFHTGESNRRVPGKGRMPWHEIGLALRDINYTGAVIMEPFVKTGGTIGSDIKVWRDLSGGADIAKMDEDARNALAFSRFVLGG

SEQ ID NO: 15 - protein, 290 aa, Pseudomonas cichorii
MNKVGMFYTYWSTEWMVDFPATAKRIAGLGFDLMEISLGEFHNLSDAKKRELKAVADDLGLTVMCCIGLKSEYDFASPDKSVRDAGTEYVKRLLDDCHLLGAPVFAGLTFCAWPQSPPLDMKDKRPYVDRAIESVRRVIKVAEDYGIIYALEVVNRFEQWLCNDAKEAIAFADAVDSPACKVQLDTFHMNIEETSFRDAILACKGKMGHFHLGEANRLPPGEGRLPWDEIFGALKEIGYDGTIVMEPFMRKGGSVSRAVGVWRDMSNGATDEEMDERARRSLQFVRDKLA